European Patent Specification EP 4 007 563 B1, published September 9, 2026. Title: Melonocyte-regulating peptides. Applicant: IDP DISCOVERY PHARMA S.L. The sequence listing filed with the application follows.

SEQUENCE LISTING (26 sequences)

SEQ ID NO: 1 - protein, 18 aa, Artificial Sequence
  Peptide
  MISC_FEATURE: the peptide comprises a linker birradical of formula (I) -[(R1)a-(R2)-(R3)b]c- connecting an amino acid at position "i" with an amino acid at position "i+3" or "i+7"
  MISC_FEATURE: R1 and R3 are birradicals independently selected from the group consisting of: (C1-C10)alkyl; (C1-C10)alkyl substituted; (C2-C10)alkenyl; (C2-C10)alkenyl substituted; (C2-C10)alkynyl; and (C2-C10)alkynyl substituted;
  MISC_FEATURE: "(C1-C10)alkyl substituted" means (C1-C10)alkyl substituted by one or more radicals selected from: halogen, (C1-C10)alkyl, OR6 ,NR7R8, SR9, SOR10, SO2R11 and CO2R12
  MISC_FEATURE: "(C2-C10)alkenyl substituted" means (C2-C10)alkenyl substituted by one or more radicals selected from: halogen, (C1-C10)alkyl, OR6 ,NR7R8, SR9, SOR10, SO2R11 and CO2R12
  MISC_FEATURE: "(C2-C10)alkynyl substituted" means (C2-C10)alkynyl substituted by one or more radicals selected from: halogen, (C1-C10)alkyl, OR6 ,NR7R8, SR9, SOR10, SO2R11 and CO2R12
  MISC_FEATURE: R2 is a birradical selected from: -O-, C(=O), C(=O)NR13, C(=O)O, S(=O), S(=O)2, NR14, (C1-C10)alkyl, (C2-C10)alkenyl, (C2-C10)alkynyl, -NR15-NR16-, -N=N-, -S-S-, and a known ring system comprising from 3 to 14 members optionally substituted
  MISC_FEATURE: "a" and "b" are the same or different and are 0 or 1; and "c" is comprised from 1 to 10
  MISC_FEATURE: the amino acids which are connected by the linker of formula (I), being of formula (II)  -NH-C(R19)-C(=O)-, wherein R19 is a monoradical selected from (C1-C10)alkyl, (C2-C10)alkenyl, (C2-C10)alkynyl and a known ring system comprising from 3 to 14
  MISC_FEATURE: the C-terminal end corresponds to -C(O)R4, wherein R4 is selected from -OH and-NR17R18
  MISC_FEATURE: the N-terminal end corresponds to -NHR5, wherein R5 is selected from -H, (C1-C20)alkyl and C1-C10)alkyl substituted by one or more radicals selected from the group consisting of: halogen, (C1-C10)alkyl, -OR6, -NR7R8, -SR9, -SOR10, -SO2R11, and -CO2R1
  MISC_FEATURE: known ring system "optionally substituted" means that the system is optionally substituted by one or more radicals independently selected from halogen,OH,NO2,(C1-C10)alkyl,(C1-C10)haloalkyl and (C1-C10)alkyl-O-
  MISC_FEATURE: R6 to R16 are radicals independently selected from H and (C1-C10)alkyl
  MISC_FEATURE: R17 to R18 are radicals independently selected from H, (C1-C10)alkyl, and (C1-C10)alkyl substituted by one or more radicals selected from the group consisting of: halogen, (C1-C10)alkyl, -OR6, -NR7R8, -SR9, -SOR10, -SO2R11, and -CO2R12
  MISC_FEATURE (1)..(1): X means (Trp)m, wherein m is 0 or 1
  MISC_FEATURE (2)..(2): X means (Asn)n, wherein n is 0 or 1
  MISC_FEATURE (17)..(17): X means (Leu)p, wherein p is 0 or 1
  MISC_FEATURE (18)..(18): X means (Gln)q, wherein q is 0 or 1
XXKGTILKASVDYIRKXX

SEQ ID NO: 2 - protein, 19 aa, Artificial Sequence
  peptide
  MISC_FEATURE: the peptide comprises a linker birradical of formula (I) -[(R1)a-(R2)-(R3)b]c- connecting an amino acid at position "i" with an amino acid at position "i+3" or "i+7"
  MISC_FEATURE: R1 and R3 are birradicals independently selected from the group consisting of: (C1-C10)alkyl; (C1-C10)alkyl substituted; (C2-C10)alkenyl; (C2-C10)alkenyl substituted; (C2-C10)alkynyl; and (C2-C10)alkynyl substituted;
  MISC_FEATURE: "(C1-C10)alkyl substituted" means (C1-C10)alkyl substituted by one or more radicals selected from: halogen, (C1-C10)alkyl, OR6,NR7R8, SR9, SOR10, SO2R11 and CO2R12
  MISC_FEATURE: "(C2-C10)alkenyl substituted" means (C2-C10)alkenyl substituted by one or more radicals selected from: halogen, (C1-C10)alkyl, OR6 ,NR7R8, SR9, SOR10, SO2R11 and CO2R12
  MISC_FEATURE: "(C2-C10)alkynyl substituted" means (C2-C10)alkynyl substituted by one or more radicals selected from: halogen, (C1-C10)alkyl, OR6 ,NR7R8, SR9, SOR10, SO2R11 and CO2R12
  MISC_FEATURE: R2 is a birradical selected from: -O-, C(=O), C(=O)NR13, C(=O)O, S(=O), S(=O)2, NR14, (C1-C10)alkyl, (C2-C10)alkenyl, (C2-C10)alkynyl, -NR15-NR16-, -N=N-, -S-S-, and a known ring system comprising from 3 to 14 members optionally substituted
  MISC_FEATURE: "a" and "b" are the same or different and are 0 or 1; and "c" is comprised from 1 to 10
  MISC_FEATURE: the amino acids which are connected by the linker of formula (I), being of formula (II) -NH-C(R19)-C(=O)-, wherein R19 is a monoradical selected from (C1-C10)alkyl, (C2-C10)alkenyl, (C2-C10)alkynyl and a known ring system comprising from 3 to 14
  MISC_FEATURE: the C-terminal end corresponds to -C(O)R4, wherein R4 is selected from -OH and-NR17R18
  MISC_FEATURE: the N-terminal end corresponds to -NHR5, wherein R5 is selected from -H, (C1-C20)alkyl, and (C1-C10)alkyl substituted by one or more radicals selected from the group consisting of: halogen, (C1-C10)alkyl, -OR6, -NR7R8, -SR9, -SOR10, -SO2R11, and -CO2R12
  MISC_FEATURE: the "known ring system" comprises from 1 to 3 rings, each one of the rings being (a) saturated, partially saturated or aromatic, and (b) isolated, partially or totally fused; and each member being selected from CH,CH2,NH,N,SH,S,and O
  MISC_FEATURE: known ring system "optionally substituted" means that the system is optionally substituted by one or more radicals independently selected from halogen,OH,NO2,(C1-C10)alkyl,(C1-C10)haloalkyl and (C1-C10)alkyl-O-
  MISC_FEATURE: R6 to R16 are radicals independently selected from H and (C1-C10)alkyl
  MISC_FEATURE: R17 to R18 are radicals independently selected from H, (C1-C10)alkyl, and (C1-C10)alkyl substituted by one or more radicals selected from the group consisting of: halogen, (C1-C10)alkyl, -OR6, -NR7R8, -SR9, -SOR10, -SO2R11, and -CO2R12
  MISC_FEATURE (1)..(1): X means (Arg)mx, wherein mx is 0 or 1
  MISC_FEATURE (2)..(2): X means (Arg)nx, wherein nx is 0 or 1
  MISC_FEATURE (18)..(18): X means (Ile)px, wherein px is 0 or 1
  MISC_FEATURE (18)..(18): X means (Pro)qx, wherein qx is 0 or 1
  misc_feature (19)..(19): Xaa can be any naturally occurring amino acid
XXRRFNINDRIKELGTLXX

SEQ ID NO: 3 - protein, 18 aa, Artificial Sequence
  peptide
  MISC_FEATURE (3)..(3): the amino acid is of formula (II), the alpha carbon of this amino acid being connected to the alpha carbon of the amino acid at position 10 by a linker "L"
  MISC_FEATURE (10)..(10): the amino acid is of formula (II), the alpha carbon of this amino acid being connected to the alpha carbon of the amino acid at position 3 by a linker "L"
  MISC_FEATURE (17)..(17): X means (Leu)p, wherein p is 0 or 1
  MISC_FEATURE (18)..(18): X means (Gln)q, wherein q is 0 or 1
WNXGTILKAXVDYIRKXX

SEQ ID NO: 4 - protein, 18 aa, Artificial Sequence
  peptide
  MISC_FEATURE (1)..(1): X means (Trp)m, wherein m is 0 or 1
  MISC_FEATURE (2)..(2): X means (Asn)n, wherein n is 0 or 1
  MISC_FEATURE (7)..(7): the amino acid is of formula (II), the alpha carbon of this amino acid being connected to the alpha carbon of amino acid at position 14 by the linker "L
  MISC_FEATURE (14)..(14): the amino acid is of formula (II), the alpha carbon of this amino acid being connected to the alpha carbon of amino acid at position 7 by the linker "L
XXKGTIXKASVDYXRKLQ

SEQ ID NO: 5 - protein, 18 aa, Artificial Sequence
  peptide
  MISC_FEATURE (1)..(1): X means (Trp)m, wherein m is 0 or 1
  MISC_FEATURE (2)..(2): X means (Asn)n, wherein n is 0 or 1
  MISC_FEATURE (10)..(10): the amino acid is of formula (II), the alpha carbon atom of this amino acid being connected to the alpha carbon of the amino acid at position 17 by linker "L"
  MISC_FEATURE (17)..(17): the amino acid is of formula (II), the alpha carbon atom of this amino acid being connected to the alpha carbon of the amino acid at position 10 by linker "L"
XXKGTILKAXVDYIRKXQ

SEQ ID NO: 6 - protein, 16 aa, Artificial Sequence
  peptide
  MISC_FEATURE (3)..(3): the amino acid is of formula (II), the alpha carbon of this amino acid being connected to the alpha carbon of amino acid at position 10 by linker "L"
  MISC_FEATURE (10)..(10): the amino acid is of formula (II), the alpha carbon of this amino acid being connected to the alpha carbon of amino acid at position 3 by linker "L"
WNXGTILKAXVDYIRK

SEQ ID NO: 7 - protein, 16 aa, Artificial Sequence
  peptide
  MISC_FEATURE (5)..(5): the amino acid is of formula (II), the alpha carbon of this amino acid being connected to the alpha carbon of the amino acid at position 12 by the linker "L"
  MISC_FEATURE (12)..(12): the amino acid is of formula (II), the alpha carbon of this amino acid being connected to the alpha carbon of the amino acid at position 5 by the linker "L"
KGTIXKASVDYXRKLQ

SEQ ID NO: 8 - protein, 16 aa, Artificial Sequence
  peptide
  MISC_FEATURE (8)..(8): the amino acid is of formula (II), the alpha carbon atom of this amino acid being connected to the alpha carbon of amino acid at position 15 by the linker "L"
  MISC_FEATURE (15)..(15): the amino acid is of formula (II), the alpha carbon atom of this amino acid being connected to the alpha carbon of amino acid at position 8 by the linker "L"
KGTILKAXVDYIRKXQ

SEQ ID NO: 9 - protein, 19 aa, Artificial Sequence
  peptide
  MISC_FEATURE (8)..(8): the amino acid is of formula (II), the alpha carbon of this amino acid being connected to the alpha carbon of amino acid at position 15 by the linker "L"
  MISC_FEATURE (15)..(15): the amino acid is of formula (II), the alpha carbon of this amino acid being connected to the alpha carbon of amino acid at position 8 by the linker "L"
  MISC_FEATURE (18)..(18): X means (Ile)px, wherein px is 0 or 1
  MISC_FEATURE (19)..(19): X means (Pro)qx, wherein qx is 0 or 1
RRRRFNIXDRIKELXTLXX

SEQ ID NO: 10 - protein, 19 aa, Artificial Sequence
  peptide
  MISC_FEATURE (1)..(1): X means (Arg)mx, wherein mx is 0 or 1
  MISC_FEATURE (2)..(2): X means (Arg)nx, wherein nx is 0 or 1
  MISC_FEATURE (6)..(6): the amino acid is of formula (II), the alpha carbon of this amino acid being connected to the alpha carbon of amino acid at position 13 by the linker "L"
  MISC_FEATURE (13)..(13): the amino acid is of formula (II), the alpha carbon of this amino acid being connected to the alpha carbon of amino acid at position 6 by the linker "L"
XXRRFXINDRIKXLGTLIP

SEQ ID NO: 11 - protein, 19 aa, Artificial Sequence
  peptide
  MISC_FEATURE (3)..(3): the amino acid is of formula (II), the alpha carbon of this amino acid being connected to the alpha carbon of amino acid at position 10 by the linker "L"
  MISC_FEATURE (10)..(10): the amino acid is of formula (II), the alpha carbon of this amino acid being connected to the alpha carbon of amino acid at position 3 by the linker "L"
  MISC_FEATURE (18)..(18): X means (Ile)px, wherein px is 0 or 1
  MISC_FEATURE (19)..(19): X means (Pro)qx, wherein qx is 0 or 1
RRXRFNINDXIKELGTLXX

SEQ ID NO: 12 - protein, 19 aa, Artificial Sequence
  peptide
  MISC_FEATURE (1)..(1): X means (Arg)mx, wherein mx is 0 or 1
  MISC_FEATURE (2)..(2): X means (Arg)nx, wherein nx is 0 or 1
  MISC_FEATURE (8)..(8): the amino acid is of formula (II), the alpha carbon of this amino acid being connected to the alpha carbon of amino acid at position 15 by the linker "L"
  MISC_FEATURE (15)..(15): the amino acid is of formula (II), the alpha carbon of this amino acid being connected to the alpha carbon of amino acid at position 8 by the linker "L"
XXRRFNIXDRIKELXTLIP

SEQ ID NO: 13 - protein, 17 aa, Artificial Sequence
  peptide
  MISC_FEATURE (8)..(8): the amino acid is of formula (II), the alpha carbon of this amino acid being connected to the alpha carbon of amino acid at position 15 by the linker "L"
  MISC_FEATURE (15)..(15): the amino acid is of formula (II), the alpha carbon of this amino acid being connected to the alpha carbon of amino acid at position 8 by the linker "L"
RRRRFNIXDRIKELXTL

SEQ ID NO: 14 - protein, 17 aa, Artificial Sequence
  peptide
  MISC_FEATURE (3)..(3): the amino acid is of formula (II), the alpha carbon atom of this amino acid being connected to the alpha carbon of amino acid at position 10 by the linker "L"
  MISC_FEATURE (10)..(10): the amino acid is of formula (II), the alpha carbon atom of this amino acid being connected to the alpha carbon of amino acid at position 3 by the linker "L"
RRXRFNINDXIKELGTL

SEQ ID NO: 15 - protein, 17 aa, Artificial Sequence
  peptide
  MISC_FEATURE (4)..(4): the amino acid is of formula (II), the alpha carbon of this amino acid being connected to the alpha carbon of amino acid at position 11 by the linker "L"
  MISC_FEATURE (11)..(11): the amino acid is of formula (II), the alpha carbon of this amino acid being connected to the alpha carbon of amino acid at position 4 by the linker "L"
RRFXINDRIKXLGTLIP

SEQ ID NO: 16 - protein, 17 aa, Artificial Sequence
  peptide
  MISC_FEATURE (6)..(6): the amino acid is of formula (II), the alpha carbon of this amino acid being connected to the alpha carbon of amino acid at position 13 by the linker "L"
  MISC_FEATURE (13)..(13): the amino acid is of formula (II), the alpha carbon of this amino acid being connected to the alpha carbon of amino acid at position 6 by the linker "L"
RRFNIXDRIKELXTLIP

SEQ ID NO: 17 - protein, 16 aa, Artificial Sequence
  peptide
  MISC_FEATURE (3)..(3): the amino acid is of formula (II), being R19 a -CH3 radical; the alpha carbon of this amino acid being connected to the alpha carbon of amino acid at position 10 by the linker -(CH2)6-CH=CH-(CH2)3-
  MISC_FEATURE (10)..(10): the amino acid is of formula (II), being R19 a -CH3 radical; the alpha carbon of this amino acid being connected to the alpha carbon of amino acid at position 3 by the linker -(CH2)6-CH=CH-(CH2)3-
WNXGTILKAXVDYIRK

SEQ ID NO: 18 - protein, 16 aa, Artificial Sequence
  peptide
  MISC_FEATURE (5)..(5): the amino acid is of formula (II) being R19 a -CH3 radical; the alpha carbon of this amino acid being connected to the alpha carbon of amino acid at position 12 by the linker -(CH2)6-CH=CH-(CH2)3-
  MISC_FEATURE (12)..(12): the amino acid is of formula (II) being R19 a -CH3 radical; the alpha carbon of this amino acid being connected to the alpha carbon of amino acid at position 5 by the linker -(CH2)6-CH=CH-(CH2)3-
KGTIXKASVDYXRKLQ

SEQ ID NO: 19 - protein, 16 aa, Artificial Sequence
  peptide
  MISC_FEATURE (8)..(8): the amino acid is of formula (II) being R19 a -CH3 radical; the alpha carbon of this amino acid being connected to the alpha carbon of amino acid at position 15 by the linker -(CH2)6-CH=CH-(CH2)3-
  MISC_FEATURE (15)..(15): the amino acid is of formula (II) being R19 a -CH3 radical; the alpha carbon of this amino acid being connected to the alpha carbon of amino acid at position 8 by the linker -(CH2)6-CH=CH-(CH2)3-
KGTILKAXVDYIRKXQ

SEQ ID NO: 20 - protein, 17 aa, Artificial Sequence
  peptide
  MISC_FEATURE (8)..(8): the amino acid is of formula (II), being R19 a -CH3 radical; the alpha carbon of this amino acid being connected to the alpha carbon of amino acid at position 15 by the linker -(CH2)6-CH=CH-(CH2)3-
  MISC_FEATURE (15)..(15): the amino acid is of formula (II), being R19 a -CH3 radical; the alpha carbon of this amino acid being connected to the alpha carbon of amino acid at position 8 by the linker -(CH2)6-CH=CH-(CH2)3-
RRRRFNIXDRIKELXTL

SEQ ID NO: 21 - protein, 17 aa, Artificial Sequence
  peptide
  MISC_FEATURE (3)..(3): the amino acid is of formula (II), being R19 a -CH3 radical; the alpha carbon of this amino acid is connected to the alpha carbon of amino acid at position 10 by the linker  -(CH2)6-CH=CH-(CH2)3-
  MISC_FEATURE (10)..(10): the amino acid is of formula (II), being R19 a -CH3 radical; the alpha carbon of this amino acid is connected to the alpha carbon of amino acid at position 4 by the linker  -(CH2)6-CH=CH-(CH2)3-
RRXRFNINDXIKELGTL

SEQ ID NO: 22 - protein, 17 aa, Artificial Sequence
  peptide
  MISC_FEATURE (4)..(4): the amino acid is of formula (II), being R19 a -CH3 radical; the alpha carbon of this amino acid being connected to the alpha carbon of amino acid  at position 11 by the linker -(CH2)6-CH=CH-(CH2)3-
  MISC_FEATURE (11)..(11): the amino acid is of formula (II), being R19 a -CH3 radical; the alpha carbon of this amino acid being connected to the alpha carbon of amino acid  at position 4 by the linker -(CH2)6-CH=CH-(CH2)3-
RRFXINDRIKXLGTLIP

SEQ ID NO: 23 - protein, 17 aa, Artificial Sequence
  peptide
  MISC_FEATURE (6)..(6): the amino acid is of formula (II), being R19 a -CH3 radical; the alpha carbon of this amino acid is connected to the alpha carbon of amino acid at position 13 by the linker  -(CH2)6-CH=CH-(CH2)3-
  MISC_FEATURE (13)..(13): the amino acid is of formula (II), being R19 a -CH3 radical; the alpha carbon of this amino acid is connected to the alpha carbon of amino acid at position 6 by the linker  -(CH2)6-CH=CH-(CH2)3-
RRFNIXDRIKELXTLIP

SEQ ID NO: 24 - protein, 16 aa, Artificial Sequence
  peptide
WNKGTILKASVDYIRK

SEQ ID NO: 25 - protein, 16 aa, Artificial Sequence
  peptide
NKGTILKASVDYIRKL

SEQ ID NO: 26 - protein, 16 aa, Artificial Sequence
  peptide
KGTILKASVDYIRKLQ